European Patent Application EP 4 124 345 A1, published February 1, 2023. Title: NANOPARTICLES FOR MUSCLE DELIVERY. Applicant: 4basebio Discovery Limited. The sequence listing filed with the application follows.

SEQUENCE LISTING (38 sequences)

SEQ ID NO: 1 - protein, 7 aa, Artificial Sequence
  Artificial Sequence
ASSLNIA

SEQ ID NO: 2 - protein, 12 aa, Artificial Sequence
  Artificial Sequence
RRQPPRSISSHP

SEQ ID NO: 3 - protein, 12 aa, Artificial Sequence
  Artificial Seqeunce
SKTFNTHPQSTP

SEQ ID NO: 4 - protein, 9 aa, Artificial Sequnece
  Artificial Sequence
CASSLNIAC

SEQ ID NO: 5 - protein, 11 aa, Artificial Sequence
  Artificial Sequence
GACASSLNIAC

SEQ ID NO: 6 - protein, 15 aa, Artificial Sequence
  Artificial Sequence
RVRRGACASSLNIAC

SEQ ID NO: 7 - protein, 31 aa, Artificial Sequence
  Artificial Sequence
KKKKKKKKKKKKKKKKRVRRGACASSLNIAC

SEQ ID NO: 8 - protein, 45 aa, Artificial Sequence
  Artificial Sequence
KKKKKKKKKKKKKKKKKKKKKKKKKKKKKKRVRRGACASSLNIAC

SEQ ID NO: 9 - protein, 27 aa, Artificial Sequence
  Artificial Sequence
KKKKKKKKKKKKKKKKGACASSLNIAC

SEQ ID NO: 10 - protein, 41 aa, Artificial Sequence
  Artificial Sequence
KKKKKKKKKKKKKKKKKKKKKKKKKKKKKKGACASSLNIAC

SEQ ID NO: 11 - protein, 9 aa, Artificial Sequence
  Artificial Sequence
GAASSLNIA

SEQ ID NO: 12 - protein, 25 aa, Artificial Sequence
  Artificial Sequence
KKKKKKKKKKKKKKKKGAASSLNIA

SEQ ID NO: 13 - protein, 39 aa, Artificial Sequence
  Artificial Sequence
KKKKKKKKKKKKKKKKKKKKKKKKKKKKKKGAASSLNIA

SEQ ID NO: 14 - protein, 14 aa, Artificial Sequence
  Artificial Sequence
CRRQPPRSISSHPC

SEQ ID NO: 15 - protein, 16 aa, Artificial Sequence
  Artificial Sequence
GACRRQPPRSISSHPC

SEQ ID NO: 16 - protein, 20 aa, Artificial Sequence
  Artificial Sequence
RVRRGACRRQPPRSISSHPC

SEQ ID NO: 17 - protein, 36 aa, Artificial Sequence
  Artificial Sequence
KKKKKKKKKKKKKKKKRVRRGACRRQPPRSISSHPC

SEQ ID NO: 18 - protein, 50 aa, Artificial Sequence
  Artificial Sequence
KKKKKKKKKKKKKKKKKKKKKKKKKKKKKKRVRRGACRRQPPRSISSHPC

SEQ ID NO: 19 - protein, 32 aa, Artificial Sequence
  Artificial Sequence
KKKKKKKKKKKKKKKKGACRRQPPRSISSHPC

SEQ ID NO: 20 - protein, 46 aa, Artificial Sequence
  Artificial Sequence
KKKKKKKKKKKKKKKKKKKKKKKKKKKKKKGACRRQPPRSISSHPC

SEQ ID NO: 21 - protein, 14 aa, Artificial Sequence
  Artificial Sequence
GARRQPPRSISSHP

SEQ ID NO: 22 - protein, 30 aa, Artificial Sequence
  Artificial Sequence
KKKKKKKKKKKKKKKKGARRQPPRSISSHP

SEQ ID NO: 23 - protein, 44 aa, Artificial Sequence
  Artificial Sequence
KKKKKKKKKKKKKKKKKKKKKKKKKKKKKKGARRQPPRSISSHP

SEQ ID NO: 24 - protein, 14 aa, Artificial Sequence
  Artificial Sequence
CSKTFNTHPQSTPC

SEQ ID NO: 25 - protein, 16 aa, Artificial Sequence
  Artificial Sequence
GACSKTFNTHPQSTPC

SEQ ID NO: 26 - protein, 20 aa, Artificial Sequence
  Artificial Sequence
RVRRGACSKTFNTHPQSTPC

SEQ ID NO: 27 - protein, 36 aa, Artificial Sequence
  Artificial Sequence
KKKKKKKKKKKKKKKKRVRRGACSKTFNTHPQSTPC

SEQ ID NO: 28 - protein, 50 aa, Artificial Sequence
  Artificial Sequence
KKKKKKKKKKKKKKKKKKKKKKKKKKKKKKRVRRGACSKTFNTHPQSTPC

SEQ ID NO: 29 - protein, 32 aa, Artificial Sequence
  Artificial Sequence
KKKKKKKKKKKKKKKKGACSKTFNTHPQSTPC

SEQ ID NO: 30 - protein, 46 aa, Artificial Sequence
  Artificial Sequence
KKKKKKKKKKKKKKKKKKKKKKKKKKKKKKGACSKTFNTHPQSTPC

SEQ ID NO: 31 - protein, 14 aa, Artificial Sequence
  Artificial Sequence
GASKTFNTHPQSTP

SEQ ID NO: 32 - protein, 30 aa, Artificial Sequence
  Artificial Sequence
KKKKKKKKKKKKKKKKGASKTFNTHPQSTP

SEQ ID NO: 33 - protein, 44 aa, Artificial Sequence
  Artificial Sequence
KKKKKKKKKKKKKKKKKKKKKKKKKKKKKKGASKTFNTHPQSTP

SEQ ID NO: 34 - protein, 4 aa, Artificial Sequence
  Artificial Sequence
RVRR

SEQ ID NO: 35 - protein, 5 aa, Artificial Sequence
  Artificial Sequence
  misc_feature (1)..(1): Xaa is c-aminocaproic acid
  misc_feature (3)..(3): Xaa is c-aminocaproic acid
XSXGG

SEQ ID NO: 36 - protein, 5 aa, Artificial Sequence
  Artifical Sequence
  misc_feature (1)..(1): Xaa is c-aminocaproic acid
  misc_feature (3)..(3): Xaa is c-aminocaproic acid
XSXGA

SEQ ID NO: 37 - DNA, 13 bp, Artificial Sequence
  Artificial Sequence
aaaaaacataaaa

SEQ ID NO: 38 - protein, 5 aa, Artificial Sequence
  Artificial Sequence
  misc_feature (1)..(1): Xaa is c-aminocaproic acid
  misc_feature (3)..(3): Xaa is c-aminocaproic acid
XSXAA